European Patent Application EP 4 159 765 A1, published April 5, 2023. Title: Bispecific antibody or antigen-binding fragment thereof and method for preparing the same. Applicant: MUSTBIO Co., Ltd. The sequence listing filed with the application follows.

SEQUENCE LISTING (9 sequences)

SEQ ID NO: 1 - protein, 450 aa, Artificial Sequence
  Heavy chain of Fc1 in PTCWT
EVQLLESGGGLVQPGGSLRLSCAASGFTFSSYIMMWVRQAPGKGLEWVSSIYPSGGITFYADTVKGRFTISRDNSKNTLYLQMNSLRAEDTAVYYCARIKLGTVTTVDYWGQGTLVTVSSASTKGPSVFPLAPSSKSTSGGTAALGCLVKDYFPEPVTVSWNSGALTSGVHTFPAVLQSSGLYSLSSVVTVPSSSLGTQTYICNVNHKPSNTKVDKKVEPKSCDKTHTCPPCPAPELLGGPSVFLFPPKPKDTLMISRTPEVTCVVVDVSHEDPEVKFNWYVDGVEVHNAKTKPREEQYNSTYRVVSVLTVLHQDWLNGKEYKCKVSNKALPAPIEKTISKAKGQPREPQVYTLPPSRDELTKNQVSLTCLVKGFYPSDIAVEWESNGQPENNYKTTPPVLDSDGSFFLYSKLTVDKSRWQQGNVFSCSVMHEALHNHYTQKSLSLSPGK

SEQ ID NO: 2 - protein, 216 aa, Artificial Sequence
  Light chain of Fc1 in PTCWT
QSALTQPASVSGSPGQSITISCTGTSSDVGGYNYVSWYQQHPGKAPKLMIYDVSNRPSGVSNRFSGSKSGNTASLTISGLQAEDEADYYCSSYTSSSTRVFGTGTKVTVLGQPKANPTVTLFPPSSEELQANKATLVCLISDFYPGAVTVAWKADGSPVKAGVETTKPSKQSNNKYAASSYLSLTPEQWKSHRSYSCQVTHEGSTVEKTVAPTECS

SEQ ID NO: 3 - protein, 232 aa, Artificial Sequence
  Fc chain of Fc2 in PTCWT
EPKSCDKTHTCPPCPAPELLGGPSVFLFPPKPKDTLMISRTPEVTCVVVDVSHEDPEVKFNWYVDGVEVHNAKTKPREEQYNSTYRVVSVLTVLHQDWLNGKEYKCKVSNKALPAPIEKTISKAKGQPREPQVYTLPPSRDELTKNQVSLTCLVKGFYPSDIAVEWESNGQPENNYKTTPPVLDSDGSFFLYSKLTVDKSRWQQGNVFSCSVMHEALHNHYTQKSLSLSPGK

SEQ ID NO: 4 - protein, 450 aa, Artificial Sequence
  Heavy chain of Fc1 in PTC019
EVQLLESGGGLVQPGGSLRLSCAASGFTFSSYIMMWVRQAPGKGLEWVSSIYPSGGITFYADTVKGRFTISRDNSKNTLYLQMNSLRAEDTAVYYCARIKLGTVTTVDYWGQGTLVTVSSASTKGPSVFPLAPSSKSTSGGTAALGCLVKDYFPEPVTVSWNSGALTSGVHTFPAVLQSSGLYSLSSVVTVPSSSLGTQTYICNVNHKPSNTKVDKKVEPKSCDKTHTCPPCPAPELLGGPSVFLFPPKPKDTLMISRTPEVTCVVVDVSHEDPEVKFNWYVDGVEVHNAKTKPREEQYNSTYRVVSVLTVLHQDWLNGKEYKCKVSNKALPAPIEKTISKAKGQPREPQVYTLPPSRDELTKNQVSLWCLVKGFYPSDIAVEWESNGQPENNYKTTPPVLDSDGSFFLYSKLTVDKSRWQQGNVFSCSVMHEALHNHYTQKSLSLSPGK

SEQ ID NO: 5 - protein, 232 aa, Artificial Sequence
  Fc chain of Fc2 in PTC019
EPKSCDKTHTCPPCPAPELLGGPSVFLFPPKPKDTLMISRTPEVTCVVVDVSHEDPEVKFNWYVDGVEVHNAKTKPREEQYNSTYRVVSVLTVLHQDWLNGKEYKCKVSNKALPAPIEKTISKAKGQPREPQVYTLPPSRDELTKNQVSLSCAVKGFYPSDIAVEWESNGQPENNYKTTPPVLDSDGSFFLVSKLTVDKSRWQQGNVFSCSVMHEALHNHYTQKSLSLSPGK

SEQ ID NO: 6 - protein, 450 aa, Artificial Sequence
  Heavy chain of Fc1 in PTC039
EVQLLESGGGLVQPGGSLRLSCAASGFTFSSYIMMWVRQAPGKGLEWVSSIYPSGGITFYADTVKGRFTISRDNSKNTLYLQMNSLRAEDTAVYYCARIKLGTVTTVDYWGQGTLVTVSSASTKGPSVFPLAPSSKSTSGGTAALGCLVKDYFPEPVTVSWNSGALTSGVHTFPAVLQSSGLYSLSSVVTVPSSSLGTQTYICNVNHKPSNTKVDKKVEPKSCDKTHTCPPCPAPELLGGPSVFLFPPKPKDTLMISRTPEVTCVVVDVSHEDPEVKFNWYVDGVEVHNAKTKPREEQYNSTYRVVSVLTVLHQDWLNGKEYKCKVSNKALPAPIEKTISKAKGQPREPQVYTFPPSRDELTKNQVSLWCLVKGFYPSDIAVEWESNGQPENNYKTTPPVLDSDGSFFLYSKLTVDKSRWQQGNVFSCSVMHEALHNHYTQKSLSLSPGK

SEQ ID NO: 7 - protein, 232 aa, Artificial Sequence
  Fc chain of Fc2 in PTC039
EPKSCDKTHTCPPCPAPELLGGPSVFLFPPKPKDTLMISRTPEVTCVVVDVSHEDPEVKFNWYVDGVEVHNAKTKPREEQYNSTYRVVSVLTVLHQDWLNGKEYKCKVSNKALPAPIEKTISKAKGQPREPQVYTGPPSRDELTKNQVSLSCAVKGFYPSDIAVEWESNGQPENNYKTTPPVLDSDGSFFLVSKLTVDKSRWQQGNVFSCSVMHEALHNHYTQKSLSLSPGK

SEQ ID NO: 8 - protein, 450 aa, Artificial Sequence
  Heavy chain of Fc1 in PTC040
EVQLLESGGGLVQPGGSLRLSCAASGFTFSSYIMMWVRQAPGKGLEWVSSIYPSGGITFYADTVKGRFTISRDNSKNTLYLQMNSLRAEDTAVYYCARIKLGTVTTVDYWGQGTLVTVSSASTKGPSVFPLAPSSKSTSGGTAALGCLVKDYFPEPVTVSWNSGALTSGVHTFPAVLQSSGLYSLSSVVTVPSSSLGTQTYICNVNHKPSNTKVDKKVEPKSCDKTHTCPPCPAPELLGGPSVFLFPPKPKDTLMISRTPEVTCVVVDVSHEDPEVKFNWYVDGVEVHNAKTKPREEQYNSTYRVVSVLTVLHQDWLNGKEYKCKVSNKALPAPIEKTISKAKGQPREPQVYTWPPSRDELTKNQVSLWCLVKGFYPSDIAVEWESNGQPENNYKTTPPVLDSDGSFFLYSKLTVDKSRWQQGNVFSCSVMHEALHNHYTQKSLSLSPGK

SEQ ID NO: 9 - protein, 232 aa, Artificial Sequence
  Fc chain of Fc2 in PTC111
EPKSCDKTHTCPPCPAPELLGGPSVFLFPPKPKDTLMISRTPEVTCVVVDVSHEDPEVKFNWYVDGVEVHNAKTKPREEQYNSTYRVVSVLTVLHQDWLNGKEYKCKVSNKALPAPIEKTISKAKGQPREPQVYTFPPSRDELTKNQVSLSCAVKGFYPSDIAVEWESNGQPENNYKTTPPVLDSDGSFFLVSKLTVDKSRWQQGNVFSCSVMHEALHNHYTQKSLSLSPGK